European Patent Application EP 4 206 327 A1, published July 5, 2023. Title: MUTANT ORF VIRUSES AND USES THEREOF. Applicant: Suzhou Prajna Biotech C0., Ltd. sequence. The sequence listing filed with the application follows.

SEQUENCE LISTING (86 sequences)

SEQ ID NO: 1 - protein, 287 aa, Artificial Sequence
  Complete sequence of the CBP protein. Amino Acid Nos: 1-16 is the signal peptide
MKAVLLLALLGAFTNAAPLLSNQRLGSAEEEKFCSTHQGEVHARFWLQMRVGVRHSPLYTPSNMCMMDIEDSTDTEDSTMEKEYTSTATGDADGLNVSVALIGEGVSIPLSYIGLRFNPSLTDGYLYVNVSSRAPWDQQTLDLSANDGWGIKQVLEKEILAIQIGCDNQKFPEEPTTTQPPSPVTTTLSSTTLDPNDENTDTTPTTTGDSVDGKRNPDDFDFSLIVDPRCVTSVNLHFEIKDACMDHKESSPLSLKGEYGDGELVRKEIKNVGKDHNMCSLNLSPGH

SEQ ID NO: 2 - protein, 271 aa, Artificial Sequence
  Mature sequence of the CBP protein
APLLSNQRLGSAEEEKFCSTHQGEVHARFWLQMRVGVRHSPLYTPSNMCMMDIEDSTDTEDSTMEKEYTSTATGDADGLNVSVALIGEGVSIPLSYIGLRFNPSLTDGYLYVNVSSRAPWDQQTLDLSANDGWGIKQVLEKEILAIQIGCDNQKFPEEPTTTQPPSPVTTTLSSTTLDPNDENTDTTPTTTGDSVDGKRNPDDFDFSLIVDPRCVTSVNLHFEIKDACMDHKESSPLSLKGEYGDGELVRKEIKNVGKDHNMCSLNLSPGH

SEQ ID NO: 3 - DNA, 1162 bp, Artificial Sequence
  Complete sequence of the ORFV112 gene
ttgctgctgctatgtcgtgcccgactctgtgcgacaaagaagcagcttaccagacgactcttcgttcatgttctctaagcaagaacactggagtgagttgccatttccgtctccaaccatataattagcatccttgtttttatcctgtatttttatcagtttttagctagttaaaacataaatagtaaagctaaaaagaggagttctggaatcttgcaacgacaggatgaaggcggtgttgttgctagcgctactgggagcgttcaccaacgcagcgcctttgttaagcaaccagcgtcttggcagtgcagaagaagaaaaattctgctcgacgcatcagggcgaagtgcacgccaggttctggcttcagatgcgcgtgggtgtacgacacagtccgctctacactcccagcaacatgtgcatgatggacatagaagactctacggacacagaagactccacgatggaaaaagaatacacgtctacggcaacgggtgatgcggacggattgaacgtgtccgtagcactaattggagaaggcgtgagcataccgctaagttacataggccttagatttaacccgtcgcttacagatggctacctgtacgtcaacgtctcgtcacgggctccttgggatcaacagactctggacctatccgcgaacgacggctggggtatcaaacaggttctagaaaaagagatactggccatccagatagggtgcgacaaccaaaaatttcccgaagaacccacaactacccaacccccctcacctgtcacaacaacgctttcctcaacaactctagatccgaatgacgaaaacacagacactacgccgacaaccaccggcgacagtgtagacggaaagcgcaatccagatgactttgacttctcgctgatcgtggacccccgatgcgtgacctctgtaaacctgcactttgagattaaggacgcgtgcatggaccacaaagaatcgtcgccgttgtcgctgaagggggaatatggagacggcgaactagtaagaaaagaaatcaaaaacgtgggaaaggatcacaatatgtgcagtcttaacctcagccctggccattgagctgtttttattcggcaatataataggtgattattgaacattaaacaaaacttatcccacaacgccgcaaca

SEQ ID NO: 4 - DNA, 624 bp, Artificial Sequence
  5' end partially deleted ORFV112 gene
ggcgtgagcataccgctaagttacataggccttagatttaacccgtcgcttacagatggctacctgtacgtcaacgtctcgtcacgggctccttgggatcaacagactctggacctatccgcgaacgacggctggggtatcaaacaggttctagaaaaagagatactggccatccagatagggtgcgacaaccaaaaatttcccgaagaacccacaactacccaacccccctcacctgtcacaacaacgctttcctcaacaactctagatccgaatgacgaaaacacagacactacgccgacaaccaccggcgacagtgtagacggaaagcgcaatccagatgactttgacttctcgctgatcgtggacccccgatgcgtgacctctgtaaacctgcactttgagattaaggacgcgtgcatggaccacaaagaatcgtcgccgttgtcgctgaagggggaatatggagacggcgaactagtaagaaaagaaatcaaaaacgtgggaaaggatcacaatatgtgcagtcttaacctcagccctggccattgagctgtttttattcggcaatataataggtgattattgaacattaaacaaaacttatcccacaacgccgcaaca

SEQ ID NO: 5 - DNA, 20 bp, Artificial Sequence
  ORFV112 gene-specific forward primer
catgcccaactgctacttcg

SEQ ID NO: 6 - DNA, 20 bp, Artificial Sequence
  ORFV112 gene-specific reverse primer
acctgtttgataccccagcc

SEQ ID NO: 7 - DNA, 42 bp, Artificial Sequence
  Forward primer for amplification of the ORFV112 gene's left arm
gaccatgattacgccaagcttcgtgatttgggaatatgcacc

SEQ ID NO: 8 - DNA, 76 bp, Artificial Sequence
  Reverse primer for amplification of theORFV112 gene's left arm
aaaataaaatttcaatttttataacttcgtatagcatacattatacgaagttatgcagcattaactgcgcgctggg

SEQ ID NO: 9 - DNA, 55 bp, Artificial Sequence
  Forward primer for amplification of the ORFV112 gene's right arm
ttttttttggaatataaatagctagcttaattaacttatcccacaacgccgcaac

SEQ ID NO: 10 - DNA, 41 bp, Artificial Sequence
  Reverse primer for amplification of the ORFV112 gene's right arm
aaaacgacggccagtgaattcgtatctatcgtcgggaccag

SEQ ID NO: 11 - DNA, 65 bp, Artificial Sequence
  Forward primer for amplification of the EGFP gene
aaaaattgaaattttattttttttttttggaatataaataaccggtcgccaccatggtgagcaag

SEQ ID NO: 12 - DNA, 100 bp, Artificial Sequence
  Reverse primer for amplification of the EGFP gene
tatttatattccaaaaaaaaaaaataaaatttcaatttttataacttcgtatagcatacattatacgaagttatacgcgttaagatacattgatgagttt

SEQ ID NO: 13 - DNA, 42 bp, Artificial Sequence; identical to SEQ ID NO: 7
  Forward primer for amplification of the linear CBP shuttle vector

SEQ ID NO: 14 - DNA, 41 bp, Artificial Sequence; identical to SEQ ID NO: 10
  Reverse primer for amplification of the linear CBP shuttle vector

SEQ ID NO: 15 - DNA, 30 bp, Artificial Sequence
  Forward primer for amplification of the px330 backbone
gtaagaattcctagagctcgctgatcagcc

SEQ ID NO: 16 - DNA, 27 bp, Artificial Sequence
  Reverse primer for amplification of the px330 backbone
tggcaccggtccaacctgaaaaaaagt

SEQ ID NO: 17 - DNA, 29 bp, Artificial Sequence
  Forward primer for amplification of Cas9 without the NLS (sequence)
ttggaccggtgccaccatggacaagaagt

SEQ ID NO: 18 - DNA, 30 bp, Artificial Sequence
  Reverse primer for amplification of Cas9 without the NLS (sequence)
ggctgatcagcgagctctaggaattcttac

SEQ ID NO: 19 - DNA, 20 bp, Artificial Sequence
  PCR identification primer 1 (OVM38F/R)-Forward primer
gagacgccgccgagcaactt

SEQ ID NO: 20 - DNA, 21 bp, Artificial Sequence
  PCR identification primer 1 (OVM38F/R)-Reverse primer
tgcagcacttcctggacatcg

SEQ ID NO: 21 - DNA, 19 bp, Artificial Sequence
  PCR identification primer 2 (OVM43F/R)-Forward primer
ggacgatcctgtgcggtag

SEQ ID NO: 22 - DNA, 20 bp, Artificial Sequence
  PCR identification primer 2 (OVM43F/R)-Reverse primer
ttgtcggcgtagtgtctgtg

SEQ ID NO: 23 - DNA, 23 bp, Artificial Sequence
  PCR identification primer 3 (OVM44F/R)-Forward primer
gatgactttgacttctcgctgat

SEQ ID NO: 24 - DNA, 20 bp, Artificial Sequence
  PCR identification primer 3 (OVM44F/R)-Reverse primer
cgacagatccatttcccaat

SEQ ID NO: 25 - DNA, 19 bp, Artificial Sequence
  PCR identification primer 4 (OVM45F/R)-Forward primer
tgcccaactgctacttcgc

SEQ ID NO: 26 - DNA, 20 bp, Artificial Sequence
  PCR identification primer 4 (OVM45F/R)-Reverse primer
caccttgatgccgttcttct

SEQ ID NO: 27 - DNA, 22 bp, Artificial Sequence
  PCR identification primer 5 (OVM46F/R)-Forward primer
agccataccacatttgtagagg

SEQ ID NO: 28 - DNA, 20 bp, Artificial Sequence
  PCR identification primer 5 (OVM46F/R)-Reverse primer
agacgatcaccagcacttcc

SEQ ID NO: 29 - DNA, 21 bp, Artificial Sequence
  PCR identification primer 6 (OVM3F2/4R2)-Forward primer
cgtgatttgggaatatgcacc

SEQ ID NO: 30 - DNA, 22 bp, Artificial Sequence
  PCR identification primer 6 (OVM3F2/4R2)-Reverse primer
gcagcattaactgcgcgctggg

SEQ ID NO: 31 - protein, 281 aa, Artificial Sequence
  Orf virus strain YX AKU76602.1
MKVVLLLVLLGALTNAAPVGNQRIDSEEKANFCSTHQNEVYARFRLQMRVGVRHSPLYVPSNMCMMDIEDSVMDNEYMSAATGDADGVNVSVALIGEGVSIPLSYIGLGFNPSLADGYLYVNVSSRAPWVQQTQDLSANGSWGIKQVLEQEMLAIQIGCDNQKFPEEPTTTQPPSPVTTTLSSTTLDSNDENADTTPPTTTSASVNRKRNSDDFDFSLLVDPRCVTSVDLHVELRDACIDYKEASLLSLKGKYGDGELVKKEIKDVGKDHNMCSLNLSPGH

SEQ ID NO: 32 - protein, 286 aa, Artificial Sequence
  Orf virus strain NA1/11AHZ33810.1
MKAVLLLALLGAFTNAAPLLESQRSNSEEKANFCSTHNNEVYARFRLQMRVGVRHSPFYTPSNMCMMDIEDSVEDIEESTEKEYASTATGEAAGVNVSVALVGEGVSIPFSYIGLGFNPSLEDSYLYVNVSSRAPWVKQTSDLSANGGWGIKQVLEKELLAIQIGCDNQKFPEEPTTTPPSPVTTTLSSTTPDLNEENTNTTPTTTSASVDRRRNLDDIDFSLLVDPRCVTSVDLHVELRDACMDYKQESPLSLKGKYGDGELVKKEIKDVGKNYNMCSLNLNPGN

SEQ ID NO: 33 - protein, 286 aa, Artificial Sequence
  Orf virus strain NZ2 ABA00630.1
MKAVLLLALLGAFTNAAPLLESQRSNSEEKANFCSTHNDEVYARFRLQMRVGVRHSPLYTPSNMCMLDIEDSVEDIEESTEKEYASTATGEAAGVNVSVALVGEGVSIPFSYIGLGFNPSLEDSYLYVNVSSRAPWVKQTSDLSANGGWGIKQVLEKELLAIQIGCDNQKFPEEPTTTPPSPVTTTLSSTTPDLNEENTENTPTTTGASVDRKRNPADDFSLLVDPRCVTSVDLHVELRDAICIDYKQESPLSLKGKYGDGELVKKEIKDVGKNHNMCSLNLNPGN

SEQ ID NO: 34 - protein, 289 aa, Artificial Sequence
  Orf virus strain NA17 AYM26053.1
MKVVVLLALLGALTNAAPVGNQRLNSKEKEDFCSTHQNEVYARFRLQMRVGVRHSPLYVPSNMCMMDIEDSVDDIEEDSIIVKEFTSTATGEAAGVNVSVALVGEGVSIPFSYIGLGFNPSLEDSYLYVNVSSRAPWVQQTPDLSANDSWGIKQVLEKELLAIQIGCDNQKFPEEPTTTQPPSLVTTTLSSTTLDLNDENTDTTPPTTTSASVNKKRNPDDFDFSLLVDPRCVTSVDLHVELRDACIDYKETSQLSLKGEYGDGELIKKEIKDVGKDHNMCSLNLNPGN

SEQ ID NO: 35 - protein, 288 aa, Artificial Sequence
  Orf virus strain OV-SA00 AAR98337.1
MKVVLLLVLLGAFTNAAPLVGNQRLDSEEKANFCSTHQNEVYARFRLQMRVGVRHSPLYTPSNMCMMDIEDSIMDIENSTEKEYTSAATGDANGVNVSVALIGEGVSIPLSYIGLGFNPSLADGYLYVNVSSRAPWVQQTLDLSANGGWGINQILEKELLAIQIGCDNQKFPEEPTTTQPPSPVTTTLSSTTLDLTDENTDTTPLTTTSASVNRKRNPDDFDFSLLVDPRCVTSVDLHVELRDACIDYKEASQLSLKGKYGDGELVKKEIKDVGKDHNMCSLNLSPGH

SEQ ID NO: 36 - protein, 286 aa, Artificial Sequence
  Orf virus strain OV-IA82 AAR98207.1
MKAAAVLLLALLGAFTNAAPVSNQRLGSEEKEKFCSTHHDEVYARFRLQMRVGVRHSPLYVPSNMCMMDIEDSTDDIEESTEKEYTSTATGEAAGVNVSVALVGEGVKIPFSYIGLGFNPSTDGYLYVNVSSRAPWVQQTPDLSANSGWGIKQVLEKELLAIQIGCDNQKFPEEPTTTPSLVTTTLSPTTTLNPNNENTDTTPTPTGASVDGKRNPDDIDFSLIVDPRCVTSVNLHFELKDACMDYKKESPLSLKGKYGDSELVKQEIKDVGKNHNMCSLNLSPGH

SEQ ID NO: 37 - protein, 280 aa, Artificial Sequence
  Orf virus strain GO AKU76734.1
MKVVLLLVLLGALTNAAPVGNQRIDSEEKANFCSTHQNEVYARFRLQMRVGVRHSPLYTPSNMCMMNIEDSMMDNEYTSTATGDADGVNVSVALMGKGVSIPLSYIGLGFNPLLADGYLYVNVSSRAPWVQQTPDLSANGGWGIKQVLEEEILAIQIGCDNQKFLEEPTTTQPPSLVTTTLSSTTLGLTDENTDTTPTTTSASVDRKRNLDDIDFSLLVDTRCVTSVNLHFEIKDACMDYKKESPLMMKGGYGDGELVRKEIKYVGTNHTMCSLNLSPGY

SEQ ID NO: 38 - protein, 280 aa, Artificial Sequence
  Orf virus strain SJ1 AKU76990.1
MKVVVLLALLGALTNAAPVGNQRLNSKEKEDFCLTHPDEVYARFRLHMRVGVRHSPLYTPSNMCMMNIEDSMMDNEYTSTATGDADGVNVSVALMGKGVSIPLSYIGLGFNPLLADGYLYVNVSSRAPWVQQTPDLSANGGWGIKQVLEEEILAIQIGCDNQKFLEEPTTPQPPSLVTTTLSSTTLGLTDENTDTTPTTTSASVDRKRNLDDIDFSLLVDTRCVTSVNLHFEIKDACMDYKKESPLMMKGGYGDGELVRKEIKYVGTNHTMCSLNLSPGY

SEQ ID NO: 39 - protein, 287 aa, Artificial Sequence
  Orf virus strain SY17 AYN61060.1
MKAVLLLALLGAFTNAAPVGNQRLDSGEKEKFCSTHQDEVYARFRLQMRVGVRHSPFYTPSNMCMMDIEDSVDDIEEDSIIVKEFTSTATGEADGVNVSVALVGEDVKIPLSYIGLGFNPSTDGYLYVNVSSRAPWVQQTLDLSANDSWGIKQVLEKELLAIQIGCDNQKFPEEPTTTQPPSLVTTTLSSTTPDLNDENTDTTPTTTGASVDRKRNPADFSFSLLVDPRCVTSVDLHVELRDACMEYKETSPLSLKGEYGDGELVKKEIKDVGKNHNMCSLNLNPGN

SEQ ID NO: 40 - protein, 286 aa, Artificial Sequence
  Orf virus strain OV-HN3/12 ASY92409.1
MKAVLLLALLGAFTNAAPLLESQRSNSEEKANFCSTHNNEVYARFRLQMRVGVRHSPFYTPSNMCMMDIEDSVEDIEESTEKEYASTATGEAAGVNVSVALVGEGVSIPFSYIGLGFNPSLEDSYLYVNVSSRAPWVKQTSDLSANGGWGIKQVLEKELLAIQIGCDNQKFPEEPTTTPPSPVTTTLSSTTPDLNEENTDTTPTTTSASVDRRRNLDDIDFSLLVDPRCVTSVDLHVELRDACMDYKQESPLSLKGKYGDGELVKKEIKDVGKNYNMCSLNLNPGN

SEQ ID NO: 41 - protein, 289 aa, Artificial Sequence
  Orf virus strain NP AKU76866.1
MKVVVLLALLGALTNAAPVGNQRLNSKEKEDFCSTHPDEVYARFRLQMRVGVRHSPLYVPSNMCMMDIEDSVDDIEEDSIIVKEFTSTATGEAAGVNVSVALVGEGVSIPFSYIGLGFNPSLEDSYLYVNVSSRAPWVQQTPDLSANDSWGIKQVLEKELLAIQIGCDNQKFPEEPTTTQPPSLVTTTLSSTTLDLNDENTDTTPPTTTSASVNKKRNPDDFDFSLLVDPRCVTSVDLHVELRDACIDYKETSQLSLKGEYGDGELIKKEIKDVGKDHNMCSLNLNPGN

SEQ ID NO: 42 - protein, 295 aa, Artificial Sequence
  Orf virus strain B029 AHH34297.1
MKAVLLLALLGAFTNAAPLLSNQRLGSAEEEKFCSTHHDKVYARFWLQMRVGVRHSSLYAPSNMCMMDIEDSTVDIEGSTETEDSTVEKEYTSAATGDANGVNVSVALMGEGVSIPLSYIGLGFNPLLKDGYLYVNVSSRAPWDQQTLDLSANDGWGIKQVLEKEILAIQIGCDNQKFPEEPTTTQPPSPVTTTLSPTTTLNPNNENTDTTPTPTGASVDGKRNPDDIDFSLIVDPRCVTSVNLHFEIKDACMDYKQESPLSLKGKYGDGELVKEEIKDVGKNHNMCSLNLSPGH

SEQ ID NO: 43 - DNA, 1069 bp, Artificial Sequence
  Orf virus strain YX KP010353.1
ttgctgctgctatatcgtacctgactctgtgttttaaagacagcagctcaccgactcttcgtccctgttctccaagcaagaacactggagtgatttgccatttccgtctccaacatataattagcatccttgtttttatcttgtctttttatcagtttttatgttagttaaaacataaatagtaaagctaaaaagagtactctggaatcttgcaacagtcaggatgaaggtggtgttgttgctagtgctactgggggcgttaaccaacgcagcgcccgtcggcaaccagcgtattgacagtgaggagaaagcaaatttctgctcgacgcatcaaaatgaagtgtacgccaggttccggcttcagatgcgcgtgggtgtacgacacagtccgctctacgttcccagcaacatgtgcatgatggacatagaagactccgtaatggataatgaatacatgtctgcggccacgggtgatgcggacggagtgaacgtgtccgtggcactaataggagaaggcgtgagcataccgctaagttacataggcctcggatttaacccatcgcttgcagatggctacctgtacgtcaacgtctcgtcacgggctccttgggttcaacagactcaagacttatctgcgaacggcagctggggtattaaacaggttctagaacaagagatgctggccatccagatagggtgcgacaaccaaaaatttcctgaagaacccacaactacccaacctccctcacctgtcacgacaacgctttcctcaacaactctagattcgaatgacgaaaacgcagacactacgccgccgaccaccaccagcgccagtgtaaacagaaagcgcaattcagatgactttgacttctcgctgctcgtagacccccgatgcgtgacctctgtagacctgcacgtcgagctcagggacgcgtgcatagactacaaagaagcgtcgctgttgtcgctgaaggggaaatatggagacggcgaactagtaaaaaaggagatcaaagacgtgggaaaggatcacaatatgtgcagtcttaacctcagccctggccattga

SEQ ID NO: 44 - DNA, 1036 bp, Artificial Sequence
  Orf virus strain NA1/11 KF234407.1
tcaacatccttgtttttatcctgtctttttatcagttttttagctagttaaaacataaatagtaaagctaaaaagaggagttctggagtcttgcaataaccaggatgaaggcggtgttgttgctggcgttactgggagcgttcaccaacgcagcgcctttgttagaaagccagcgttctaacagtgaggagaaagcaaatttctgctcgacgcataataatgaagtgtacgccaggttcaggcttcagatgcgcgtgggtgtacgacacagtcctttctacactcccagcaacatgtgcatgatggacatagaagactccgttgaggacatagaagagtccacagagaaagaatacgcgtctacggccacgggtgaggcggccggagtgaacgtgtcagtggcactagtgggagaaggcgtgagcataccgtttagttacataggccttggattcaacccgtcgcttgaagatagctacctgtacgttaacgtctcgtcacgagctccttgggttaaacagacttcggacctatccgcgaacggcggctggggtattaaacaggttctagaaaaagagttactggccatccaaatagggtgcgacaaccaaaaatttcccgaagaacccacaactacacccccctcacctgtcacgacaacgctttcctcaacaactccagatctgaatgaagaaaacacaaacactacgccgacgaccaccagcgccagtgtagacagaaggcgcaatctagatgacattgacttctcgctgctcgtggacccccgatgcgtgacctctgtagacctacacgtcgagctcagggacgcgtgcatggactacaaacaagagtcgccgttgtcgctgaaggggaaatatggagacggcgagctagtaaaaaaggagatcaaagacgtgggaaagaattacaatatgtgcagtcttaacctcaaccctggcaattgagatgtttttattcggcaatataatagggattattgaacattaaacaaaacttatcccacaacgccgcaaca

SEQ ID NO: 45 - DNA, 1036 bp, Artificial Sequence
  Orf virus strain NZ2 DQ184476.1
tcagcatccttgtttttatcctgtctttttatcagttttttagctagttaaaacataaatagtaaagctaaaaagaggagttctggagtcttgcaacaaccaggatgaaggcggtgttgttgctggcgttactgggagcgttcaccaacgcagcgcctttgttagaaagccagcgttctaacagtgaggaaaaagcaaatttctgctcgacgcataatgatgaagtgtacgccaggttcaggcttcagatgcgcgtgggtgtacgacacagtccgctctacactcccagcaacatgtgcatgctggacatagaagactccgttgaggacatagaagagtccacagaaaaagaatacgcgtctacggccacgggtgaggcggccggagtgaacgtgtcagtggcactagtgggagaaggcgtgagcataccgtttagttacataggccttggattcaacccgtcgcttgaagatagctacctgtacgtcaacgtctcgtcacgagctccttgggttaaacagacttcggacctatccgcgaacggcggctggggtatcaaacaggttctagaaaaagagttactggccatccaaatagggtgcgacaaccaaaaatttcccgaagaacccacaactacacccccctcacctgtcactacaacgctttcctcaacaactccagatctgaatgaagaaaacacagaaaatacgccgacgaccaccggcgccagtgtagacagaaagcgcaatccagctgacattgacttctcgctgctcgtggacccccgatgcgtgacctctgtagacctgcacgtcgagctcagggacgcgtgcatagactacaaacaagagtcgccgttgtcgctgaaggggaaatatggagacggcgaactagtaaaaaaggagattaaagacgtgggaaagaatcacaatatgtgcagtcttaacctcaaccctggcaattgagctgtttttattcggcaatataataggtgattattgaacattaaacaaaacttatcccacaacgccgcaac

SEQ ID NO: 46 - DNA, 1166 bp, Artificial Sequence
  Orf virus strain NA17 MG674916.2
ttgctgctgctatatcgtacctgactctgtgttacaaagacagcagctcaccagactcttcgtccctgttctctaagcaagaacactggagtgagttgccatttccgtctccaacatataattagcatccttgtttttatcttgtctttttatcagtttttatgctagttaaaacataaatagtaaagctaaaaagagtactctggaatcttgcaacaatcaggatgaaggtggtggtgttgctggcgctactgggagcgttaaccaacgcagcgcccgtcggcaaccagcgtcttaacagtaaagagaaagaagatttctgctcgacgcatcaaaatgaagtgtacgccaggttccggcttcagatgcgcgtgggtgtacgacacagtccgctctacgttcccagcaacatgtgcatgatggacatagaagactctgttgatgacatagaagaagactccattatagtaaaagaattcacgtctacagccacgggtgaggcggccggagtgaacgtgtccgtggcactagtgggagaaggcgtgagcataccgtttagttacataggccttggattcaacccgtcgcttgaagatagctacttgtacgtcaacgtctcgtcacgagctccttgggttcaacagactccagacttatctgcaaacgacagctggggtattaaacaggttctagaaaaagagttactggccatccaaatagggtgcgacaaccaaaaatttcccgaagaacccacaaccacccaacccccctcacttgtcacgacaacgctttcctcaacaactctagatctgaatgacgaaaacacagacactacgccgccaaccaccaccagcgccagcgtaaacaaaaagcgcaatccagatgactttgacttctcgctgctcgtggacccccgatgcgtgacctctgtagacctgcacgtcgagctcagggacgcgtgcatagactacaaagaaacgtcgcagttgtcgctgaagggggaatatggagacggcgaactaataaaaaaggagatcaaagacgtgggaaaggatcacaatatgtgcagtcttaacctcaaccctggcaattgagctgtttttattcggcaatataataggtgattattgaacattaaacaaaacttatcccacaacgccgcaaca

SEQ ID NO: 47 - DNA, 1161 bp, Artificial Sequence
  Orf virus strain OV-SA00 AY386264.1
ttgctgcgctatgtcgtgcccgactctgtgcgacaaagacagaagctcaccaaactcttcgtctctgttctccaagcaagaacactggagtgatttgccatttccgtctccaacatataattagcatccttgtttttatcttgtctttttatcagtttttatgttagttaaaacataaatagtaaagctaaaaagagtactctggaatcttgcaacagtcaggatgaaggtggtgttgttgctagtgctactgggagcgtttaccaacgcagcgcctttggtcggcaaccagcgtcttgacagtgaggagaaagcaaatttctgctcgacacatcaaaatgaagtgtacgccaggttccggcttcagatgcgcgtgggtgtacgacacagtccgctctacactcccagcaacatgtgcatgatggacatagaagactccattatggacatagaaaactccacagaaaaagaatacacgtctgcagccacgggtgatgcgaacggagtgaacgtgtccgtggcactaataggagaaggcgtgagcataccgctaagttacataggcctcggattcaacccatcgcttgcagatggctacctgtacgtcaacgtctcgtcacgagctccttgggttcaacagactctagacctatccgcgaacggcggctggggtattaatcagattctagaaaaagagttactggccatccaaatagggtgcgacaaccaaaaatttcccgaagaacccacaactacccaacctccctcacctgtcacgacaacgctttcctcaacaacgctagatctgactgacgaaaacacagacactacgccgctgaccaccaccagcgccagtgtaaacagaaagcgcaatccagatgactttgacttctcgctgctcgtggacccccgatgcgtgacctctgtagacttgcacgtcgagctcagggacgcgtgcatagactacaaagaagcgtcgcagttgtcgctgaaggggaaatatggagacggcgaactagtaaaaaaggagatcaaagacgtgggaaaggatcacaatatgtgcagtcttaacctcagccctggccattgagatgtttttattcggcaattaataggtgattattgaacattaaacaaaacttatcccacaacgccgcaaca

SEQ ID NO: 48 - DNA, 1159 bp, Artificial Sequence
  Orf virus strain OV-IA82 AY386263.1
ttgctgctgctatgtcgtgcccgactctgtgcgacaaagacagcggctaaccagactcttcgtccctgttctccaagcaaaaaactggagtgagttgccatttccgtctccaaccatataattagcatccttgtttttatcctgtatttttatcagtttttatgctagttaaaacataaatagtaaggctaaaaagaagagttctagaatcttgcaacaaccaagatgaaggcggcggcggtgttgttgctagcgctactgggagcgttcaccaacgcagcgcccgtcagcaaccagcgtcttggcagtgaggagaaagaaaaattctgctcgactcatcatgacgaagtgtacgccaggttccggcttcagatgcgcgtgggtgtacgacacagtccgctctacgttcccagcaacatgtgcatgatggacatagaagactctacggatgacatagaagagtccacggagaaagaatacacgtctacggctacgggtgaggcggccggagtgaacgtgtccgtggcactagtgggagaaggcgtgaaaataccgtttagttacataggccttggattcaacccatctacagatggctacctgtacgtcaacgtctcgtcacgagctccttgggttcaacagactccagacctatccgcgaacagcggctggggtattaaacaggttctagaaaaagagttactggccatccagatagggtgcgacaaccaaaaatttcccgaagaacccacaactaccccctcacttgtcacgacaacgctttccccaacaacgactttaaatccgaataacgaaaacacagacactacgccgacgcccaccggcgccagtgtagacggaaagcgcaatccagatgacattgacttctcgctgatcgtggacccccgatgcgtgacctctgtaaacctgcacttcgagctcaaggacgcgtgcatggactacaaaaaagagtcgccgttgtcgctgaaggggaaatatggagacagtgaactagtaaaacaggagattaaagacgtgggaaagaatcacaatatgtgcagtcttaacctcagccctggccattgagctgtttttattcggcaatataataaggtgattattgaacattaaacaaaacttatcccacaacgccgcaaca

SEQ ID NO: 49 - DNA, 1138 bp, Artificial Sequence
  Orf virus strain GO KP010354.1
ttgctgcgctatgtcgtgcccgactctgtgcgacaaagacagaagctcaccaaactcttcgtctctgttctccaagcaagaacactggagtgatttgccatttccgtctccaacatataattagcatccttgtttttatcttgtctttttatcagtttttatgttagttaaaacataaatagtaaagctaaaaagagtactctggaatcttgcaacagtcaggatgaaggtggtgttgttgctagtgctactgggggcgttaaccaacgcagcgcccgtcggcaaccagcgtattgacagtgaggagaaagcaaatttctgctcgacgcatcaaaatgaagtgtacgccaggttccggcttcagatgcgcgtgggtgtacggcacagtccgctctacactcccagcaacatgtgcatgatgaacatagaagactccatgatggataatgaatacacgtctacggccacaggtgatgcggacggagtgaacgtgtctgtggcactaatgggaaaaggcgtgagcataccgttaagttacataggcctcggattcaacccattgcttgcagatggctacctgtacgtcaacgtctcgtcacgagctccttgggttcaacaaactccggacctatccgcgaacggcggctggggtattaaacaggttctagaagaagagatactggccatccagatagggtgcgacaaccaaaaatttctagaagaacccacaacaacccaacccccctcacttgtcacgacaacgctttcctcaacaacgctaggtctgactgacgagaacacagacactacgccgacgaccaccagcgccagtgtagacagaaagcgcaatctagatgacattgacttctcgctgctcgtagacacccgatgcgtgacctcggtaaacctgcacttcgagattaaggacgcgtgtatggactacaaaaaagagtcgccgttgatgatgaaggggggatatggagacggcgaactagtaagaaaagagatcaaatacgtgggaacgaatcacactatgtgcagtctcaacctcagccctggctattgatttgtttttattcggcaatataataggtgattattgaacattaaacaaaacttatcccacaacgcctcaaca

SEQ ID NO: 50 - DNA, 1138 bp, Artificial Sequence
  Orf virus strain SJ1 KP010356.1
ttgctgcgctatgtcgtgcccgactctgtgcgacaaagacagaagctcaccaaactcttcgtctctgttctccaagtaagaacactggagtgatttgccatttccgtctccaacatataattagcatccttgtttttatcttgtctttttatcagtttttatgctagttaaaacataaatagtaaagctaaaaagagtactctggaatcttgcaacagtcaggatgaaggtggtggtgttgctggcgctactgggagcgttaaccaacgcagcgcccgttggcaaccagcgtcttaacagtaaagagaaagaagatttctgcttgacgcatccggatgaagtgtatgccaggttccggcttcatatgcgcgtgggtgtacgacacagtccgctttacactcccagcaacatgtgcatgatgaacatagaagactccatgatggataatgaatacacgtctacggccacgggtgatgcggacggagtgaacgtgtctgtggcactaatgggaaaaggcgtgagcataccgttaagttacataggcctaggattcaacccattgcttgcagatggctacttgtacgtcaacgtctcgtcacgagctccttgggttcaacagactccggacctatccgcgaacggcggctggggtattaaacaggttctagaagaagagatactggccatccagatagggtgcgacaaccaaaaatttctagaagaacccacaactccccaacccccctcacttgtcacgacaacgctttcctcaacaacgctaggtctgactgacgagaacacagacactacgccgacgaccaccagcgccagtgtagacagaaagcgcaatctagatgacattgacttctcgctgctcgtagacacccgatgcgtgacctcggtaaacctgcacttcgagatcaaggacgcgtgtatggactacaaaaaagagtcgccgttgatgatgaaggggggatatggagacggcgaactagtaagaaaagagatcaaatacgtgggaacgaatcacactatgtgcagtctcaacctcagccctggctattgatttgtttttattcggcaatataataggtgattattgaacattaaacaaaacttatcccacaacgccgcaaca

SEQ ID NO: 51 - DNA, 1040 bp, Artificial Sequence
  Orf virus strain SY17 MG712417.1
tcagcatccttgtttttatcctgtctttttatcagttttttagctagttaaaacataaatagtaaagctaaaaagaggagttctggagtcttgtaacaaccaggatgaaggcggtgttgttgctggcgttactgggagcgttcactaacgcagcgcccgtcggcaaccagcgtctcgatagtggggagaaagaaaaattctgctcgacgcatcaggatgaagtgtacgctaggttcaggcttcagatgcgcgtgggtgtacgacacagtcctttctacactcccagcaacatgtgcatgatggacatagaagactccgttgatgacatagaagaagactccattatagtaaaagaatttacgtctacggccacgggtgaggcggacggagtgaacgtgtccgtggcactagtgggagaagacgtgaaaataccgttaagttacataggccttggattcaacccatctacagatggctacctgtacgtcaacgtctcgtcacgagctccttgggttcaacagactctagacctatctgcgaacgacagctggggtattaaacaggttctagaaaaagagttactggccatccaaatagggtgcgacaaccaaaaatttcctgaagaacccacaaccacccaacctccctcacttgtcacgacaacgctttcctcaacaactccagatctgaatgacgaaaacacagacactacgccgacgaccactggcgccagtgtagacagaaagcgcaatccagctgactttagtttctcgctgctcgtggacccccgatgcgtgacttctgtagacctgcacgtcgagctcagggacgcgtgcatggagtacaaagaaacgtcgccgttgtcgctgaagggggaatatggagacggcgaactagtaaaaaaggagatcaaagacgtgggaaagaatcacaatatgtgcagtcttaacctcaaccctggcaattaagctgtttttattcggcaatataataggtgattattgaacattaaacaaaacttatcccacaacgccgcaaca

SEQ ID NO: 52 - DNA, 1035 bp, Artificial Sequence
  Orf virus strain OV-HN3/12 KY053526.1
tcaacatccttgtttttatcctgtctttttatcagtttttagctagttaaaacataaatagtaaagctaaaaagaggagttctggagtcttgcaataaccaggatgaaggcggtgttgttgctggcgttactgggagcgttcaccaacgcagcgcctttgttagaaagccagcgttctaacagtgaggagaaagcaaatttctgctcgacgcataataatgaagtgtacgccaggttcaggcttcagatgcgcgtgggtgtacgacacagtcctttctacactcccagcaacatgtgcatgatggacatagaagactccgttgaggacatagaagagtccacagagaaagaatacgcgtctacggccacgggtgaggcggccggagtgaacgtgtcagtggcactagtgggagaaggcgtgagcataccgtttagttacataggccttggattcaacccgtcgcttgaagatagctacctgtacgttaacgtctcgtcacgagctccttgggttaaacagacttcggacctatccgcgaacggcggctggggtattaaacaggttctagaaaaagagttactggccatccaaatagggtgcgacaaccaaaaatttcccgaagaacccacaactacacccccctcacctgtcacgacaacgctttcctcaacaactccagatctgaatgaagaaaacacagacactacgccgacgaccaccagcgccagtgtagacagaaggcgcaatctagatgacattgacttctcgctgctcgtggacccccgatgcgtgacctctgtagacctacacgtcgagctcagggacgcgtgcatggactacaaacaagagtcgccgttgtcgctgaaggggaaatatggagacggcgagctagtaaaaaaggagatcaaagacgtgggaaagaattacaatatgtgcagtcttaacctcaaccctggcaattgagatgtttttattcggcaatataatagggattattgaacattaaacaaaacttatcccacaacgccgcaaca

SEQ ID NO: 53 - DNA, 1163 bp, Artificial Sequence
  Orf virus strain NP KP010355.1
ttgctgcgctatgtcgtacctgactctgtgtacaaagacagcagctcaccagactcttcgtccctgttctctaagcaagaacactggagtgagttgccatttccgtctccgacatataattagcatccttgtttttatcctgtctttttatcagtttttatgctagttaaaacataaatagtaaagctaaaaagagtactctggaatcttgcaacaatcaggatgaaggtggtggtgttgctggcgctactgggagcgttaaccaacgcagcgcccgtcggcaaccagcgtcttaacagtaaagagaaagaagatttctgctcgacgcatccggatgaagtgtacgccaggttccggcttcagatgcgcgtgggtgtacgacacagtccgctctacgttcccagcaacatgtgcatgatggacatagaagactctgttgatgacatagaagaagactccattatagtaaaagaattcacgtctacagccacgggtgaggcggccggagtgaacgtgtccgtggcactagtgggagaaggcgtgagcataccgtttagttacataggccttggattcaacccgtcgcttgaagatagctacttgtacgtcaacgtctcgtcacgagctccttgggttcaacagactccagacttatctgcaaacgacagctggggtattaaacaggttctagaaaaagagttactggccatccaaatagggtgcgacaaccaaaaatttcccgaagaacccacaaccacccaacccccctcacttgtcacgacaacgctttcctcaacaactctagatctgaatgacgaaaacacagacactacgccgccaaccaccaccagcgccagcgtaaacaaaaagcgcaatccagatgactttgacttctcgctgctcgtggacccccgatgcgtgacctctgtagacctgcacgtcgagctcagggacgcgtgcatagactacaaagaaacgtcgcagttgtcgctgaagggggaatatggagacggcgaactaataaaaaaggagatcaaagacgtgggaaaggatcacaatatgtgcagtcttaacctcaaccctggcaattgagctgtttttattcggcgtataataggtgattattgaacattaaacaaaacttatcccacaacgccgcaaca

SEQ ID NO: 54 - DNA, 1183 bp, Artificial Sequence
  Orf virus strain B029 KF837136.1
ttgctgctatgtcgtacccgactctgtgctacaaagacagcagctcaccagactcttcgtccctgttctccaagcaagaacactggagtgagttgccatttccgtctccaaccatataattagcatccttgtttttatcctgtatttttatcagtttttatgctagttaaaacataaatagtaaggctaaaaagaagagttctagaatcttgcaacaaccaagatgaaggcggtgttgttgctagcgctactgggagcgttcaccaacgcagcgcctttgttaagcaaccagcgtcttggcagtgcagaggaagaaaaattctgctcgacgcatcatgacaaagtgtacgccaggttctggcttcagatgcgtgtgggtgtacgacacagttcgctctacgctcccagcaacatgtgcatgatggacatagaagactctacggtggacatagaaggctccacggaaacagaagactccacggtggaaaaagaatacacgtctgcggcaacgggtgatgcgaacggagtgaacgtgtccgtggcactaatgggagaaggcgtgagcataccgctaagttacataggcctcggattcaacccattgcttaaagatggctacctgtacgtcaacgtctcgtcacgggctccttgggatcaacagactctggacctatccgcgaacgacggctggggtattaaacaggttctagaaaaagagatactggccatccagatagggtgcgacaaccaaaaatttcccgaagaacccacaactacccaacccccctcacctgtcacaacaacgctttccccaacaacgactttaaacccgaataacgaaaacacagacactacgccgacgcccaccggcgccagtgtagacggaaagcgcaatccagatgacattgacttctcgctgatcgtggacccccgatgcgtgacctctgtaaacctgcacttcgagatcaaggacgcgtgcatggactacaaacaagagtcgccgttgtcgctgaaggggaaatatggagacggtgaactagtaaaagaggagattaaagacgtgggaaagaaccacaatatgtgcagtcttaacctcagccctggccattgagctgtttttattcggcaatataataggtgattattgaacattaaacaaaacttatcccacaacgccgcaaca

SEQ ID NO: 55 - DNA, 21 bp, Artificial Sequence
  Forward primer
cgtgatttgggaatatgcacc

SEQ ID NO: 56 - DNA, 20 bp, Artificial Sequence
  Reverse primer
gtatctatcgtcgggaccag

SEQ ID NO: 57 - DNA, 22 bp, Artificial Sequence
  5'truncated ORFV112 gene
cttatcccacaacgccgcaaca

SEQ ID NO: 58 - protein, 179 aa, Artificial Sequence
  Full peptide sequence of the hypothetical protein 111
MSRLQILTSFGQIYAPDEARLREIARDLGICTIKRAFGDMLYGFIDFNPVPLTQVNMLMPNCYFAVNGNLLPCTEDFRLRLPATEISAAYLTKTGRTILCGRDFNIVAPSGFKPSMRLRNLSHVSALVEILELYDESGEYQFVLGPSAQLMLRLMEKENVCLFGRGWCIVDLRKLDVAI

SEQ ID NO: 59 - DNA, 794 bp, Artificial Sequence
  Full DNA sequence of the ORFV111 gene
aaatatactgtttgaacgcaaagacgccatgtcgcgacttcaaatactgacctcatttggacaaatctacgcacctgacgaagctcggctgcgagagatcgcgcgtgatttgggaatatgcaccataaaacgcgcattcggcgacatgctgtacggctttatagacttcaacccggtgcccctgacccaagtaaacatgctcatgcccaactgctacttcgcggtcaacggcaacctgcttccgtgcacggaggacttccggctcagactcccggcaacggagatctctgcggcctacctgacgaaaacgggacggacgatcctgtgcggtagagacttcaacatagtagcgccgtcggggttcaagccgtccatgcggctgcgcaacctcagtcacgtgtctgcgcttgtagagattttagagctttacgacgagtccggagagtaccaattcgtgctcggccccagcgcgcagttaatgctgcggctaatggagaaggagaatgtctgtctgtttggcagaggttggtgcatagtggacctgcgcaagctggacgtagccatataattgctgctgctatgtcgtgcccgactctgtgcgacaaagaagcagcttaccagacgactcttcgttcatgttctctaagcaagaacactggagtgagttgccatttccgtctccaaccatataattagcatccttgtttttatcctgtatttttatcagtttttagctagttaaaacataaatagtaaagctaaaaagaggagttctggaatcttgcaacgacagg

SEQ ID NO: 60 - DNA, 485 bp, Artificial Sequence
  3' truncated type of the ORFV111 gene
aaatatactgtttgaacgcaaagacgccatgtcgcgacttcaaatactgacctcatttggacaaatctacgcacctgacgaagctcggctgcgagagatcgcgcgtgatttgggaatatgcaccataaaacgcgcattcggcgacatgctgtacggctttatagacttcaacccggtgcccctgacccaagtaaacatgctcatgcccaactgctacttcgcggtcaacggcaacctgcttccgtgcacggaggacttccggctcagactcccggcaacggagatctctgcggcctacctgacgaaaacgggacggacgatcctgtgcggtagagacttcaacatagtagcgccgtcggggttcaagccgtccatgcggctgcgcaacctcagtcacgtgtctgcgcttgtagagattttagagctttacgacgagtccggagagtaccaattcgtgctcggccccagcgcgcagttaatgctgc

SEQ ID NO: 61 - protein, 179 aa, Artificial Sequence
  Orf virus strain YX AKU76601.1
MSQLQILTSFGQIYAPDEARLREIARDLGICTIKRAFGDMLYGFIDFNPVPLTQVNMLMSDFYFAVNGNLLPCTEDFRLRLPATDISAAYLTKTGRTILCGKDFNIVAPSGFKPSMRLRNLSHVSALVEILEFYSESGEYQFVLGPSAQFMLRLMEKENVCLFGSGWCIVDLRKLDVTI

SEQ ID NO: 62 - protein, 179 aa, Artificial Sequence
  Orf virus strain NA1/11 AHZ33809.1
MSRLQILTSFGQIYAPDEARLREIARDLGVCTIKRAFGDMLYGFIDFDPVPLTQVNMLMPNCYFAVNGNLLPCTEDFRLRLPATEISAAYLTRTGRTILCGKDFNIVAPSGFKPSMRLRDLSHVSALVEILEIYNESGEYQFVLGPSAQFMLRLMEKENVCLFGSGWCIVDLRKLDVPI

SEQ ID NO: 63 - protein, 179 aa, Artificial Sequence
  Orf virus strain NZ2 ABA00629.1
MSRLQILTSFGQIFAPDEARLREIARDLGICTIKRAFGDMLYGFIDFDPVPLTQVNMLMSNCYFAVNGNLLPCTEDFRLRLPATEISAAYLTRTGRTILCGKDFNIVAPSGFKPSMRLRDLSHVSALVEILEVYDESGEYQFVLGPSAQFMLRLMEKENVCLFGSGWCIVDLRKLDVPI

SEQ ID NO: 64 - protein, 179 aa, Artificial Sequence
  Orf virus strain NA17 AYM26052.1
MSRLQILTSFGQIYAPDEARLREIARDLGICTIKRAFGDMLYGFIDFNPVPLTQVNMLMSDCYFAVNGNLLPCTEDFRLRLPATEISAAYLTKTGRTILCGKDFNIIAPSGFKPSMRLRNLSHVSALVEILEFYSESGEYQFVLGPSAQFMLRLMEKENVCLFGSGWCIVDLRKLDVTI

SEQ ID NO: 65 - protein, 179 aa, Artificial Sequence
  Orf virus strain OV-SA00 AAR98336.1
MSRLQILTSFGQIYAPDEARLREIARDLGICTIKRAFGDMLYGFIDFNPVPLTQVNMLMSNCYFAVNGNLLPCTEDFRLRLPATEISAAYLTKTGRTILCGKDFNIIAPLGFKPSMRLRNLSHVSALVEILEFYSESGEYQFVLGPSAQFMLRLMEKENVCLFGSGWCIVDLRKLDVTI

SEQ ID NO: 66 - protein, 198 aa, Artificial Sequence
  Orf virus strain OV-IA82 AAR98206.1
MHEGDARITENILFERKDAMSRLQILTSFGQIYAPDEARLREIARDLGICTIKRAFGDMLYGFIDFNPVPLTQVNMLMSNCYFAVNGNLLPCTEDFRLRLPATEISAAYLTRTGRTILCGKDFNIVAPSGFKPSMRLRDLSHVSALVEILELYDESGDYQFVLGPSAQFMLRLMEKENVCLFGNGWCIVDLRKLDVTI

SEQ ID NO: 67 - protein, 179 aa, Artificial Sequence; identical to SEQ ID NO: 64
  Orf virus strain GO AKU76733.1

SEQ ID NO: 68 - protein, 179 aa, Artificial Sequence
  Orf virus strain SJ1 AKU76989.1
MSQLQILTSFGQIYAPDEARLREIARDLGICTIKRAFGDMLYGFIDFNPVPLTQVNMLMSNCYFAVNGNLLPCTEDFRLRLPATEISAAYLTKTGRTILCGKDFNIVAPSGFKPSMRLRNLSHVSALVEILEFYSESGEYQFVLGPSAQFMLRLMEKENVCLFGSGWCIVDLRKLDVTI

SEQ ID NO: 69 - protein, 179 aa, Artificial Sequence
  Orf virus strain SY17 AYN61059.1
MSRLQILTSFGQIYAPDEARLREIARDLGICTIKRAFGDMLYGFIDFNPVPLTQVNMLMPNCYFAVNGNLLPCTEDFRLRLPATEISAAYLTRTGRTILCGKDFNIVAPSGFKPSMRLRDLSHVSALVEILEIYNESGEYQFVLGPSAQFMLRLMEKENVCLFGSGWCIVDLRKLDVTI

SEQ ID NO: 70 - protein, 179 aa, Artificial Sequence; identical to SEQ ID NO: 62
  Orf virus strain OV-HN3/12 ASY92408.1

SEQ ID NO: 71 - protein, 179 aa, Artificial Sequence
  Orf virus strain NP AKU76865.1
MSRLQILTSFGQIYAPDEARLREIARDLGICTIKRAFGDMLYGFIDFNPVPLTQVNMLMSDFYFAVNGNLLPCTEDFRLRLPATDISAAYLTKTGRTILCGKDFNIVAPSGFKPSMRLRNLSHVSALVEILEFYSESGEYQFVLGPSAQFMLRLMEKENVCLFGSGWCIVDLRKLDVTI

SEQ ID NO: 72 - protein, 179 aa, Artificial Sequence
  Orf virus strain B029 AIO03573.1
MSRLQILTSFGQIYAPDEARLREIARDLGICTIKRAFGDMLYGFIDFNPVPLTQVNMLMSNCYFAVNGNLLPCTEDFRLRLPATEISAAYLTKTGRTILCGKDFNIVAPSGFKPSMRLRDLSHVSALVEILELYDESGEYQFVLGPSAQFMLRLMEKENVCLFGNGWCIVDLRKLDVTI

SEQ ID NO: 73 - DNA, 795 bp, Artificial Sequence
  Orf virus strain YX KP010353.1
ctgaaaatatactgtttgaatgcaaagacgccatgtcgcaacttcaaatactgacctcatttggacaaatctacgcacccgacgaagctcggctgcgcgagatcgcgcgtgatttgggaatatgcaccataaaacgcgcattcggcgacatgctgtacggctttatagacttcaacccggtgccccttacccaagtaaacatgctcatgtccgacttctacttcgcggtcaacggcaacctgcttccgtgcacggaggacttccggctcagactcccggcgacggatatctctgcggcctacctgacgaaaacgggacggacgatcctgtgcggcaaagacttcaacatagtggcgccgtcagggttcaagccgtccatgcggctgcgcaacctcagtcacgtgtctgcgcttgtagagatcttggagttttacagcgagtccggggagtaccaattcgtgctcggccccagcgcgcagttcatgctgcggctgatggagaaggagaacgtctgtctgttcggcagcggatggtgcatagtggacctgcgcaagctggacgtaaccatataattgctgctgctatatcgtacctgactctgtgttttaaagacagcagctcaccgactcttcgtccctgttctccaagcaagaacactggagtgatttgccatttccgtctccaacatataattagcatccttgtttttatcttgtctttttatcagtttttatgttagttaaaacataaatagtaaagctaaaaagagtactctggaatcttgcaacagtcagg

SEQ ID NO: 74 - DNA, 675 bp, Artificial Sequence
  Orf virus strain NA1/11 KF234407.1
ctgaaaatatactgtttgaacgcaaagacgccatgtcgcgacttcaaatactgacctcatttggacaaatctacgcacccgacgaagctcggctgcgcgagatcgcgcgtgatttgggagtatgcaccataaaacgcgcattcggcgacatgctgtacggctttatagacttcgacccggttcccctgacccaagtaaacatgctcatgcccaactgctacttcgcggttaacggcaacctgcttccgtgcacggaggacttcaggctcagactcccggcaacggagatctccgcggcctacctgacgagaacgggacggacgatcctgtgcggcaaagacttcaacatagtggcgccgtcagggttcaagccgtccatgcggctgcgcgaccttagtcacgtgtctgcgcttgtagagatcctggaaatctacaacgagtccggggagtaccaattcgtgctcggccccagcgcgcagttcatgctgcggctgatggagaaggaaaacgtctgtctgttcggcagcgggtggtgcatagtggacctgcgcaagctggacgtacccatatatcaacatccttgtttttatcctgtctttttatcagttttttagctagttaaaacataaatagtaaagctaaaaagaggagttctggagtcttgcaataaccagg

SEQ ID NO: 75 - protein, 676 aa, Artificial Sequence
  Orf virus strain NZ2 DQ184476.1
CTGAAAATATACTGTTTGAACGCAAAGACGCCATGTCGCGACTTCAAATACTGACCTCATTTGGACAAATCTTCGCACCCGACGAAGCTCGGCTGCGCGAGATCGCGCGTGATTTGGGAATATGCACCATAAAACGCGCATTCGGCGACATGCTGTACGGCTTTATAGACTTCGACCCGGTGCCCCTGACCCAAGTAAACATGCTCATGTCCAACTGCTACTTCGCGGTCAACGGCAACCTGCTTCCGTGCACGGAGGACTTCCGGCTCAGACTCCCGGCAACGGAGATCTCTGCGGCCTACCTGACGAGAACGGGACGGACGATCCTGTGCGGCAAAGACTTCAACATAGTAGCGCCGTCGGGGTTCAAGCCGTCCATGCGGCTGCGCGACCTCAGTCACGTGTCTGCGCTTGTAGAGATCCTGGAAGTCTACGACGAGTCCGGGGAGTACCAATTCGTGCTCGGCCCCAGCGCGCAGTTCATGCTGCGGCTGATGGAGAAGGAGAACGTCTGTCTGTTCGGCAGCGGGTGGTGCATAGTGGACCTGCGCAAGCTGGACGTACCCATATAATCAGCATCCTTGTTTTTATCCTGTCTTTTTATCAGTTTTTTAGCTAGTTAAAACATAAATAGTAAAGCTAAAAAGAGGAGTTCTGGAGTCTTGCAACAACCAGG

SEQ ID NO: 76 - protein, 796 aa, Artificial Sequence
  Orf virus strain NA17 MG674916.2
CTGAAAATATACTGTTTGAACGCAAAGACGCCATGTCGCGACTTCAAATACTGACCTCATTTGGACAAATCTACGCACCCGACGAAGCTCGGCTGCGCGAGATCGCGCGTGACTTGGGAATATGCACCATAAAACGCGCATTCGGCGACATGCTGTACGGCTTTATAGACTTCAACCCGGTGCCCCTTACCCAAGTAAACATGCTCATGTCCGACTGCTACTTCGCGGTCAACGGCAACCTGCTTCCGTGCACGGAGGACTTCCGGCTCAGACTCCCGGCGACGGAGATCTCCGCGGCCTACCTGACGAAAACGGGACGGACGATCCTGTGCGGCAAAGACTTCAACATAATAGCGCCGTCGGGTTTCAAGCCGTCCATGCGGCTGCGCAACCTCAGTCACGTGTCTGCGCTTGTAGAGATCTTGGAGTTTTACAGCGAGTCCGGGGAGTACCAATTCGTGCTCGGCCCCAGCGCGCAGTTCATGCTGCGGCTGATGGAGAAGGAAAACGTCTGTCTGTTTGGCAGCGGTTGGTGCATAGTGGACCTGCGCAAGCTGGACGTAACCATATAATTGCTGCTGCTATATCGTACCTGACTCTGTGTTACAAAGACAGCAGCTCACCAGACTCTTCGTCCCTGTTCTCTAAGCAAGAACACTGGAGTGAGTTGCCATTTCCGTCTCCAACATATAATTAGCATCCTTGTTTTTATCTTGTCTTTTTATCAGTTTTTATGCTAGTTAAAACATAAATAGTAAAGCTAAAAAGAGTACTCTGGAATCTTGCAACAATCAGG

SEQ ID NO: 77 - DNA, 791 bp, Artificial Sequence
  Orf virus strain OV-SA00 AY386264.1
aaatatactgtttgaacgcaaagacgccatgtcgcgacttcaaatactgacctcatttggacaaatctacgcacccgacgaagctcggctgcgcgagatcgcgcgtgacttgggaatatgcaccataaaacgcgcattcggcgacatgctgtacggctttatagacttcaacccggtgcccctgacccaagtaaacatgctcatgtccaactgttacttcgcggtcaacggcaacctgcttccgtgcacggaggacttccggctcagactcccggcgacggagatctctgcggcctacctgacgaaaacgggacggacgatcctgtgcggcaaagacttcaacataatagcgccgttggggttcaagccgtccatgcggctgcgcaacctcagtcacgtgtctgcgcttgtagagatcttggagttttacagcgagtccggggagtaccaatttgtgctcggccccagcgcgcagttcatgctgcgtctgatggagaaggagaacgtctgtctgttcggcagcggttggtgcatagtggacctgcgcaagctagacgtaactatataattgctgcgctatgtcgtgcccgactctgtgcgacaaagacagaagctcaccaaactcttcgtctctgttctccaagcaagaacactggagtgatttgccatttccgtctccaacatataattagcatccttgtttttatcttgtctttttatcagtttttatgttagttaaaacataaatagtaaagctaaaaagagtactctggaatcttgcaacagtcagg

SEQ ID NO: 78 - DNA, 822 bp, Artificial Sequence
  Orf virus strain OV-IA82 AY386263.1
atgcatgaaggagatgcacggataactgaaaatatactgtttgaacgcaaagacgccatgtcgcgacttcaaatactgacctcatttggacaaatctacgcacccgacgaagctcggctgcgcgagatcgcgcgtgatttgggaatatgcaccataaaacgcgcattcggcgacatgctgtacggctttatagacttcaacccggtgcccctgacccaagtaaacatgctcatgtccaactgctacttcgcggtcaacggcaacctgcttccgtgcacggaggacttccggctcagactcccggcaacggagatctctgcggcctacctgacgagaacgggacggacgatcctgtgcggcaaagacttcaacatagtggcgccgtcagggttcaagccgtccatgcggctgcgcgaccttagtcacgtgtctgcgcttgtagagatcctggagctctacgacgagtccggggattaccaattcgtgctcggccccagcgcgcagttcatgctgcggctgatggagaaggagaatgtctgtctgttcggcaacggttggtgcatagtggacctgcgcaagctagacgtaaccatataattgctgctgctatgtcgtgcccgactctgtgcgacaaagacagcggctaaccagactcttcgtccctgttctccaagcaaaaaactggagtgagttgccatttccgtctccaaccatataattagcatccttgtttttatcctgtatttttatcagtttttatgctagttaaaacataaatagtaaggctaaaaagaagagttctagaatcttgcaacaaccaag

SEQ ID NO: 79 - DNA, 791 bp, Artificial Sequence
  Orf virus strain GO KP010354.1
aaatatactgtttgaacgcaaagacgccatgtcgcgacttcaaatactgacctcatttggacaaatctacgcacccgacgaagctcggctgcgcgagatcgcgcgtgacttgggaatatgcaccataaaacgcgcattcggcgacatgctgtacggctttatagacttcaacccggtgccccttacccaagtaaacatgctcatgtctgactgctacttcgcggtcaacggcaacctgcttccgtgcacggaggacttccggctcagactcccggcgacggagatctccgcggcctacctgacgaaaacgggacggacgatcctgtgcggcaaagacttcaacataatagcgccgtcgggtttcaagccgtccatgcggctgcgcaacctcagtcacgtgtctgcgcttgtagaaatcttggagttttacagcgagtccggggagtaccaattcgtgctcggccccagcgcgcagttcatgctgcggctgatggagaaggagaatgtctgtctgttcggcagcggttggtgcatagtggacctgcgcaagctagacgtaaccatataattgctgcgctatgtcgtgcccgactctgtgcgacaaagacagaagctcaccaaactcttcgtctctgttctccaagcaagaacactggagtgatttgccatttccgtctccaacatataattagcatccttgtttttatcttgtctttttatcagtttttatgttagttaaaacataaatagtaaagctaaaaagagtactctggaatcttgcaacagtcagg

SEQ ID NO: 80 - DNA, 795 bp, Artificial Sequence
  Orf virus strain SJ1 KP010356.1
ctgaaaatatactgtttgaatgcaaagacgccatgtcgcaacttcaaatactgacctcatttggacaaatctacgcacccgacgaagctcggctgcgcgagatcgcgcgtgatttgggaatatgcaccataaaacgcgcattcggcgacatgctgtacggctttatagacttcaacccggtgccccttacccaagtaaacatgctcatgtccaactgctacttcgcagtcaacggcaacctgcttccgtgcacggaggacttccggctcagactcccggcgacggagatctctgcggcctacctgacgaaaacgggacggacgatcctgtgcggcaaagacttcaacatagtggcgccgtcggggttcaagccgtccatgcggctgcgcaacctcagtcacgtgtctgcgcttgtagagatcttggagttttacagcgagtccggggagtaccaattcgtgctcggccccagcgcgcagttcatgctgcggctgatggagaaggagaatgtctgtctgttcggcagcggttggtgcatagtggacctgcgcaagctagacgtaaccatataattgctgcgctatgtcgtgcccgactctgtgcgacaaagacagaagctcaccaaactcttcgtctctgttctccaagtaagaacactggagtgatttgccatttccgtctccaacatataattagcatccttgtttttatcttgtctttttatcagtttttatgctagttaaaacataaatagtaaagctaaaaagagtactctggaatcttgcaacagtcagg

SEQ ID NO: 81 - DNA, 676 bp, Artificial Sequence
  Orf virus strain SY17 MG712417.1
ctgaaaatatactgtttgaacgcaaagacgccatgtcgcgacttcaaatactgacctcatttggacaaatctacgcacccgacgaagctcggctgcgcgagatcgcgcgtgatttgggaatatgcaccataaaacgcgcattcggcgacatgctgtacggctttatagacttcaacccggtgcccctgacccaagtaaacatgctcatgcccaactgctacttcgctgtcaacggcaacctgcttccgtgcacggaggacttccggcttagactcccggcaacggagatctctgcggcctacctaacgagaacgggacggacgatcctgtgcggcaaagacttcaacatagtggcgccgtcagggttcaagccgtccatgcggctgcgcgacctcagtcacgtgtctgcgcttgtagagatcctggaaatctacaacgagtccggggagtaccaattcgtgctcggccccagcgcgcagttcatgctgcggctgatggagaaggaaaacgtctgtctgttcggcagcgggtggtgcatagtggacctgcgcaagctggacgtaaccatataatcagcatccttgtttttatcctgtctttttatcagttttttagctagttaaaacataaatagtaaagctaaaaagaggagttctggagtcttgtaacaaccagg

SEQ ID NO: 82 - DNA, 675 bp, Artificial Sequence
  Orf virus strain OV-HN3/12 KY053526.1
ctgaaaatatactgtttgaacgcaaagacgccatgtcgcgacttcaaatactgacctcatttggacaaatctacgcacccgacgaagctcggctgcgcgagatcgcgcgtgatttgggagtatgcaccataaaacgcgcattcggcgacatgctgtacggctttatagacttcgacccggttcccctgacccaagtaaacatgctcatgcccaactgctacttcgcggttaacggcaacctgcttccgtgcacggaggacttcaggctcagactcccggcaacggagatctccgcggcctacctgacgagaacgggacggacgatcctgtgcggcaaagacttcaacatagtggcgccgtcagggttcaagccgtccatgcggctgcgcgaccttagtcacgtgtctgcgcttgtagagatcctggaaatctacaacgagtccggggagtaccaattcgtgctcggccccagcgcgcagttcatgctgcggctgatggagaaggaaaacgtctgtctgttcggcagcgggtggtgcatagtggacctgcgcaagctggacgtacccatataatcaacatccttgtttttatcctgtctttttatcagtttttagctagttaaaacataaatagtaaagctaaaaagaggagttctggagtcttgcaataaccagg

SEQ ID NO: 83 - DNA, 794 bp, Artificial Sequence
  Orf virus strain NP KP010355.1
ctgaaaatatactgtttgaacgcaaagacgccatgtcgcgacttcaaatactgacctcatttggacaaatctacgcacccgacgaagctcggctgcgcgagatcgcgcgtgacttgggaatatgcaccataaaacgcgcattcggcgacatgctgtacggctttatagacttcaacccggtgccccttacccaagtaaacatgctcatgtccgacttctacttcgcggtcaacggcaacctgcttccgtgcacggaggacttccggctcagactcccggcgacggatatctctgcggcctacctgacgaaaacgggacggacgatcctgtgcggcaaagacttcaacatagtggcgccgtcagggttcaagccgtccatgcggctgcgcaacctcagtcacgtgtctgcgcttgtagagatcttggagttttacagcgagtccggggagtaccaatttgtgctcggccccagcgcgcagttcatgctgcggctgatggagaaggagaacgtctgtctgttcggcagcggttggtgcatagtggacctgcgcaagctagacgtaaccatataattgctgcgctatgtcgtacctgactctgtgtacaaagacagcagctcaccagactcttcgtccctgttctctaagcaagaacactggagtgagttgccatttccgtctccgacatataattagcatccttgtttttatcctgtctttttatcagtttttatgctagttaaaacataaatagtaaagctaaaaagagtactctggaatcttgcaacaatcagg

SEQ ID NO: 84 - DNA, 790 bp, Artificial Sequence
  Orf virus strain B029 KF837136.1
aaatatactgtttgaacgcaaagacaccatgtcgcgacttcaaatactgacctcatttggacaaatctacgcacccacgaagctcggctgcgcgagatcgcgcgtgatttgggaatatgcaccataaaacgcgcattcggcgacatgctgtacggctttatagacttcaacccggtgcccctgacccaagtaaacatgctcatgtccaactgctacttcgcggtcaacggcaacctgcttccgtgcacggaggacttccggctcagactcccggcaacggagatctctgcagcctacctgacgaaaacgggacggacgatcctgtgcggcaaagacttcaacatagtggcgccgtcggggttcaagccgtccatgcggctgcgcgacctcagtcacgtgtctgcgcttgtagagatcctggagctctacgacgagtccggggagtaccaattcgtgctcggccccagcgcgcagttcatgctgcggctgatggagaaggagaatgtctgtctgttcggcaacgggtggtgcatagtggacctgcgcaagctagacgtaaccatataattgctgctatgtcgtacccgactctgtgctacaaagacagcagctcaccagactcttcgtccctgttctccaagcaagaacactggagtgagttgccatttccgtctccaaccatataattagcatccttgtttttatcctgtatttttatcagtttttatgctagttaaaacataaatagtaaggctaaaaagaagagttctagaatcttgcaacaaccaag

SEQ ID NO: 85 - protein, 154 aa, Artificial Sequence
  Amino acid sequence of the ORFV111 gene of the POV-601-1A1 strain (mutant)
MSRLQILTSFGQIYAPDEARLREIARDLGICTIKRAFGDMLYGFIDFNPVPLTQVNMLMPNCYFAVNGNLLPCTEDFRLRLPATEISAAYLTKTGRTILCGRDFNIVAPSGFKPSMRLRNLSHVSALVEILELYDESGEYQFVLGPSAQLMLRR

SEQ ID NO: 86 - protein, 183 aa, Artificial Sequence
  Amino acid sequence of the ORFV112 gene of the POV-601-1A1 strain (mutant)
GVSIPLSYIGLRFNPSLTDGYLYVNVSSRAPWDQQTLDLSANDGWGIKQVLEKEILAIQIGCDNQKFPEEPTTTQPPSPVTTTLSSTTLDPNDENTDTTPTTTGDSVDGKRNPDDFDFSLIVDPRCVTSVNLHFEIKDACMDHKESSPLSLKGEYGDGELVRKEIKNVGKDHNMCSLNLSPGH